European Patent Specification EP 3 760 738 B1, published October 9, 2024. Title: Multiplex PCR amplification method for species and human individual recognition and identification of unknown biological sample suspected to be from human. Applicant: NINGBO HEALTH GENE TECHNOLOGIES CO., LTD. The sequence listing filed with the application follows.

SEQUENCE LISTING (54 sequences)

SEQ ID NO: 1 - DNA, 22 bp, Artificial Sequence
ccctgggctctgtaaagaatag

SEQ ID NO: 2 - DNA, 21 bp, Artificial Sequence
actggtggtaggaactgtaaa

SEQ ID NO: 3 - DNA, 21 bp, Artificial Sequence
gccacacggcctggcaactta

SEQ ID NO: 4 - DNA, 25 bp, Artificial Sequence
gtcctgtagattattttcactgtgg

SEQ ID NO: 5 - DNA, 26 bp, Artificial Sequence
aggaggtagatagactggatagatag

SEQ ID NO: 6 - DNA, 23 bp, Artificial Sequence
ctcaattccccaagtgaattgcc

SEQ ID NO: 7 - DNA, 21 bp, Artificial Sequence
gctgtagtctcagctacttgc

SEQ ID NO: 8 - DNA, 23 bp, Artificial Sequence
gactggtgtgtggagatgtctta

SEQ ID NO: 9 - DNA, 25 bp, Artificial Sequence
ttcttccctgtctcaccccttttcc

SEQ ID NO: 10 - DNA, 26 bp, Artificial Sequence
cgagtggaggtgcctaaagacttcat

SEQ ID NO: 11 - DNA, 26 bp, Artificial Sequence
caatctaaaagtttcacttagagtcc

SEQ ID NO: 12 - DNA, 26 bp, Artificial Sequence
caataggagctgtagccaccgaccta

SEQ ID NO: 13 - DNA, 21 bp, Artificial Sequence
ggttttcaagcgctcggatgc

SEQ ID NO: 14 - DNA, 20 bp, Artificial Sequence
acctccgaataaacctgggg

SEQ ID NO: 15 - DNA, 22 bp, Artificial Sequence
gaactgtggctcatctatgaaa

SEQ ID NO: 16 - DNA, 25 bp, Artificial Sequence
gctaagtggctgtggtgttatgata

SEQ ID NO: 17 - DNA, 27 bp, Artificial Sequence
catagccacagtttacaacatttgtat

SEQ ID NO: 18 - DNA, 26 bp, Artificial Sequence
tgacaagggtgattttcctctttggt

SEQ ID NO: 19 - DNA, 28 bp, Artificial Sequence
gtaagaattataacgattccacatttat

SEQ ID NO: 20 - DNA, 28 bp, Artificial Sequence
tataaagggtatgatagaacacttgtca

SEQ ID NO: 21 - DNA, 26 bp, Artificial Sequence
gtgcttacagatggcatattgtgaaa

SEQ ID NO: 22 - DNA, 27 bp, Artificial Sequence
gcccacttctaaaacacctctaatgtt

SEQ ID NO: 23 - DNA, 24 bp, Artificial Sequence
gaagtgagccatgatcacaccact

SEQ ID NO: 24 - DNA, 24 bp, Artificial Sequence
tagaagtactttctcttagcctgt

SEQ ID NO: 25 - DNA, 22 bp, Artificial Sequence
gagcagctgagtggccaaatcc

SEQ ID NO: 26 - DNA, 22 bp, Artificial Sequence
agctcgagggcactgcggtaaa

SEQ ID NO: 27 - DNA, 23 bp, Artificial Sequence
caaatcaacagaggcttgcatgt

SEQ ID NO: 28 - DNA, 23 bp, Artificial Sequence
gtgacagagcaagaccctgtctc

SEQ ID NO: 29 - DNA, 19 bp, Artificial Sequence
ccgattatccagcctggcc

SEQ ID NO: 30 - DNA, 21 bp, Artificial Sequence
ggctctggggtgattcccatt

SEQ ID NO: 31 - DNA, 26 bp, Artificial Sequence
tgttggttacatgaataagttcttta

SEQ ID NO: 32 - DNA, 24 bp, Artificial Sequence
tgaggctgcaaaaagctataattg

SEQ ID NO: 33 - DNA, 25 bp, Artificial Sequence
cagggaagatgaaaaaagagactgt

SEQ ID NO: 34 - DNA, 25 bp, Artificial Sequence
gattttggcttttagacctggactg

SEQ ID NO: 35 - DNA, 26 bp, Artificial Sequence
gctcatctctacaaactcaggggctt

SEQ ID NO: 36 - DNA, 25 bp, Artificial Sequence
ctatttccctgcaccgttttgtcct

SEQ ID NO: 37 - DNA, 20 bp, Artificial Sequence
cagccctgggatcctgctca

SEQ ID NO: 38 - DNA, 26 bp, Artificial Sequence
gaataaaatctccctggttgcaagca

SEQ ID NO: 39 - DNA, 19 bp, Artificial Sequence
cagaacaggcacttaggga

SEQ ID NO: 40 - DNA, 25 bp, Artificial Sequence
gctttctgtccttgtcagcgtttat

SEQ ID NO: 41 - DNA, 21 bp, Artificial Sequence
agatcccaagctcttcctctt

SEQ ID NO: 42 - DNA, 21 bp, Artificial Sequence
ctgtgtgcatctgtaagcatg

SEQ ID NO: 43 - DNA, 22 bp, Artificial Sequence
tcaaatctcctccttcaacttg

SEQ ID NO: 44 - DNA, 24 bp, Artificial Sequence
gagttcatttctttagtgggcatc

SEQ ID NO: 45 - DNA, 23 bp, Artificial Sequence
acttcaattctgcttctcagatc

SEQ ID NO: 46 - DNA, 28 bp, Artificial Sequence
actcacagattaaactgtaaccaaaata

SEQ ID NO: 47 - DNA, 26 bp, Artificial Sequence
ctgccttcatagatagaagatagata

SEQ ID NO: 48 - DNA, 24 bp, Artificial Sequence
ctcagaccctgttctaagtacttc

SEQ ID NO: 49 - DNA, 27 bp, Artificial Sequence
gtggatgataagaataatcagtatgtg

SEQ ID NO: 50 - DNA, 30 bp, Artificial Sequence
attttggacagatgataaatacataggatg

SEQ ID NO: 51 - DNA, 27 bp, Artificial Sequence
gattctccttcagtcctgtgttagtca

SEQ ID NO: 52 - DNA, 23 bp, Artificial Sequence
ggtggtagagatggaagaaaatc

SEQ ID NO: 53 - DNA, 29 bp, Artificial Sequence
gatgtgtgtaaagtgcttagtatcatgat

SEQ ID NO: 54 - DNA, 25 bp, Artificial Sequence
tgaaaaattagctgggtgtggtggt